European Patent Specification EP 4 105 654 B1, published October 22, 2025. Title: Method for detecting contents of whey protein and casein, and/or ratio thereof in milk powder. Applicant: Beijing Sanyuan Foods Co., Ltd. The sequence listing filed with the application follows.

SEQUENCE LISTING (4 sequences)

SEQ ID NO: 1 - protein, 8 aa, Bovine
  PEPTIDE (1)..(8)
LDQWLCEK

SEQ ID NO: 2 - protein, 7 aa, Bovine
  PEPTIDE (1)..(7)
VLPVPQK

SEQ ID NO: 3 - protein, 11 aa, Bovine
  PEPTIDE (1)..(11)
TPEVDDEALEK

SEQ ID NO: 4 - protein, 8 aa, Bovine
  PEPTIDE (1)..(8)
FALPQYLK